European Patent Application EP 4 793 361 A1, published August 19, 2026. Title: PROCESSO IN VITRO PARA DIAGNÓSTICO E/OU PROGNÓSTICO DE TUMORES EM AMOSTRAS LÍQUIDAS, KIT E PROCESSO IN VITRO PARA MONITORAMENTO DO QUADRO CLÍNICO. Applicant: LIQSCI BIOTECNOLOGIA LTDA. Application BR, filed October 9, 2023. The sequence listing filed with the application follows.

SEQUENCE LISTING (19 sequences)

SEQ ID NO: 1 - DNA, 21 bp, synthetic construct
  source 1..21: mol_type = other DNA
gtgtaccctaactagccgagg

SEQ ID NO: 2 - DNA, 20 bp, synthetic construct
  source 1..20: mol_type = other DNA
ggctgtgtcgactgaggaaa

SEQ ID NO: 3 - DNA, 20 bp, synthetic construct
  source 1..20: mol_type = other DNA
cctgcttggtgctgatttgt

SEQ ID NO: 4 - DNA, 20 bp, synthetic construct
  source 1..20: mol_type = other DNA
aagccaagatccactaccgg

SEQ ID NO: 5 - DNA, 23 bp, synthetic construct
  source 1..23: mol_type = other DNA
tgaggacctctgtgtatttgtca

SEQ ID NO: 6 - DNA, 20 bp, synthetic construct
  source 1..20: mol_type = other DNA
gaaacaggccgagaagaacg

SEQ ID NO: 7 - DNA, 23 bp, synthetic construct
  source 1..23: mol_type = other DNA
ccacctagaatctgctggctact

SEQ ID NO: 8 - DNA, 20 bp, synthetic construct
  source 1..20: mol_type = other DNA
gggtccaaggatttggtgtg

SEQ ID NO: 9 - DNA, 20 bp, synthetic construct
  source 1..20: mol_type = other DNA
acttgaagatggtgatcgct

SEQ ID NO: 10 - DNA, 28 bp, synthetic construct
  source 1..28: mol_type = other DNA
acagacagatttgtcatgaagaaactca

SEQ ID NO: 11 - DNA, 23 bp, synthetic construct
  source 1..23: mol_type = other DNA
ggagatacgtagggagagaggaa

SEQ ID NO: 12 - DNA, 19 bp, synthetic construct
  source 1..19: mol_type = other DNA
catgagagtggagtatcac

SEQ ID NO: 13 - DNA, 16 bp, synthetic construct
  source 1..16: mol_type = other DNA
accccaaggccaaccg

SEQ ID NO: 14 - DNA, 22 bp, synthetic construct
  source 1..22: mol_type = other DNA
agcctggatagcaacgtacatg

SEQ ID NO: 15 - DNA, 18 bp, synthetic construct
  source 1..18: mol_type = other DNA
aagatgacccagatcatg

SEQ ID NO: 16 - DNA, 25 bp, synthetic construct
  source 1..25: mol_type = other DNA
ttgaggacctctgtgtatttgtcaa

SEQ ID NO: 17 - DNA, 23 bp, synthetic construct
  source 1..23: mol_type = other DNA
cctggaggagaagaggaaagaga

SEQ ID NO: 18 - DNA, 20 bp, synthetic construct
  source 1..20: mol_type = other DNA
aggtacttgagggggactgg

SEQ ID NO: 19 - DNA, 20 bp, synthetic construct
  source 1..20: mol_type = other DNA
aaatcatgccaggtcagacg